European Patent Specification EP 3 491 024 B1, published December 18, 2024. Title: ANTI-IDIOTYPIC ANTIBODIES AND RELATED METHODS. Applicant: Juno Therapeutics, Inc. HAUSKINS, Colin HEIPEL, Mark D. SUTHERLAND, Claire L. SATHALIYA, Taher SMITH, Jeff. Application Not Yet Assigned. The sequence listing filed with the application follows.

SEQUENCE LISTING (164 sequences)

SEQ ID NO: 1 - protein, 122 aa, Artificial Sequence
  anti-ID VH
QVQLQQPGSELVRPGGSVKLSCKASDYTFTSYWMHWVRQRPGQGLEWIGNIYPGSGGTNYDEKFKRKATLTVDTSSSTAYMQLRSLTSEDSAVYYCTREVTTVAYYYSMDYWGQGTSVTVSS

SEQ ID NO: 2 - protein, 324 aa, Artificial Sequence
  anti-ID CH
AKTTPPSVYPLAPGSAAQTNSMVTLGCLVKGYFPEPVTVTWNSGSLSSGVHTFPAVLQSDLYTLSSSVTVPSSTWPSETVTCNVAHPASSTKVDKKIVPRDCGCKPCICTVPEVSSVFIFPPKPKDVLTITLTPKVTCVVVDISKDDPEVQFSWFVDDVEVHTAQTQPREEQFNSTFRSVSELPIMHQDWLNGKEFKCRVNSAAFPAPIEKTISKTKGRPKAPQVYTIPPPKEQMAKDKVSLTCMITDFFPEDITVEWQWNGQPAENYKNTQPIMDTDGSYFVYSKLNVQKSNWEAGNTFTCSVLHEGLHNHHTEKSLSHSPGK

SEQ ID NO: 3 - protein, 446 aa, Artificial Sequence
  anti-ID heavy chain
QVQLQQPGSELVRPGGSVKLSCKASDYTFTSYWMHWVRQRPGQGLEWIGNIYPGSGGTNYDEKFKRKATLTVDTSSSTAYMQLRSLTSEDSAVYYCTREVTTVAYYYSMDYWGQGTSVTVSSAKTTPPSVYPLAPGSAAQTNSMVTLGCLVKGYFPEPVTVTWNSGSLSSGVHTFPAVLQSDLYTLSSSVTVPSSTWPSETVTCNVAHPASSTKVDKKIVPRDCGCKPCICTVPEVSSVFIFPPKPKDVLTITLTPKVTCVVVDISKDDPEVQFSWFVDDVEVHTAQTQPREEQFNSTFRSVSELPIMHQDWLNGKEFKCRVNSAAFPAPIEKTISKTKGRPKAPQVYTIPPPKEQMAKDKVSLTCMITDFFPEDITVEWQWNGQPAENYKNTQPIMDTDGSYFVYSKLNVQKSNWEAGNTFTCSVLHEGLHNHHTEKSLSHSPGK

SEQ ID NO: 4 - protein, 19 aa, Artificial Sequence
  anti-ID HC signal sequence
MGWSSIILFLVATASGVHS

SEQ ID NO: 5 - protein, 107 aa, Artificial Sequence
  anti-ID VL
DIQMTQTTSSLSASLGDRVTISCRASQDISNYLNWYQQKPDGTVKLLIYYTSRLHSGVPSRFSGSGSGTDYSLTISNLEQEDIATYFCQQGKTVPFTFGSGTKLEIK

SEQ ID NO: 6 - protein, 107 aa, Artificial Sequence
  anti-ID CL
RADAAPTVSIFPPSSEQLTSGGASVVCFLNNFYPKDINVKWKIDGSERQNGVLNSWTDQDSKDSTYSMSSTLTLTKDEYERHNNYTCEATHKTSTSPIVKSFNRNEC

SEQ ID NO: 7 - protein, 214 aa, Artificial Sequence
  anti-ID light chain
DIQMTQTTSSLSASLGDRVTISCRASQDISNYLNWYQQKPDGTVKLLIYYTSRLHSGVPSRFSGSGSGTDYSLTISNLEQEDIATYFCQQGKTVPFTFGSGTKLEIKRADAAPTVSIFPPSSEQLTSGGASVVCFLNNFYPKDINVKWKIDGSERQNGVLNSWTDQDSKDSTYSMSSTLTLTKDEYERHNNYTCEATHKTSTSPIVKSFNRNEC

SEQ ID NO: 8 - protein, 20 aa, Artificial Sequence
  anti-ID LC signal sequence
MMSSAQFLGLLLLCFQGTRC

SEQ ID NO: 9 - protein, 5 aa, Artificial Sequence
  anti-ID HC-CDR1
SYWMH

SEQ ID NO: 10 - protein, 17 aa, Artificial Sequence
  anti-ID HC-CDR2
NIYPGSGGTNYDEKFKR

SEQ ID NO: 11 - protein, 13 aa, Artificial Sequence
  anti-ID HC-CDR3
EVTTVAYYYSMDY

SEQ ID NO: 12 - protein, 11 aa, Artificial Sequence
  anti-ID LC-CDR1
RASQDISNYLN

SEQ ID NO: 13 - protein, 7 aa, Artificial Sequence
  anti-ID LC-CDR2
YTSRLHS

SEQ ID NO: 14 - protein, 9 aa, Artificial Sequence
  anti-ID LC-CDR3
QQGKTVPFT

SEQ ID NO: 15 - DNA, 366 bp, Artificial Sequence
  anti-ID VH
caggtccaactgcaacaacctgggtctgagctggtgaggcctggaggttcagtgaagctgtcctgcaaggcttctgactacactttcaccagctactggatgcactgggtgaggcagaggcctggacaaggccttgagtggattggaaatatttatcctggtagtggtggtactaactacgatgagaagttcaagaggaaggccacactgactgtagacacatcctccagcacagcctacatgcagctccgcagcctgacatctgaggactctgcggtctattactgtacaagagaggttactacagtagcttattactattctatggactactggggtcaaggaacctcagtcaccgtctcctca

SEQ ID NO: 16 - DNA, 975 bp, Artificial Sequence
  anti-ID CH
gccaaaacgacacccccatctgtctatccactggcccctggatctgctgcccaaactaactccatggtgaccctgggatgcctggtcaagggctatttccctgagccagtgacagtgacctggaactctggatccctgtccagcggtgtgcacaccttcccagctgtcctgcagtctgacctctacactctgagcagctcagtgactgtcccctccagcacctggcccagcgagaccgtcacctgcaacgttgcccacccggccagcagcaccaaggtggacaagaaaattgtgcccagggattgtggttgtaagccttgcatatgtacagtcccagaagtatcatctgtcttcatcttccccccaaagcccaaggatgtgctcaccattactctgactcctaaggtcacgtgtgttgtggtagacatcagcaaggatgatcccgaggtccagttcagctggtttgtagatgatgtggaggtgcacacagctcagacgcaaccccgggaggagcagttcaacagcactttccgctcagtcagtgaacttcccatcatgcaccaggactggctcaatggcaaggagttcaaatgcagggtcaacagtgcagctttccctgcccccatcgagaaaaccatctccaaaaccaaaggcagaccgaaggctccacaggtgtacaccattccacctcccaaggagcagatggccaaggataaagtcagtctgacctgcatgataacagacttcttccctgaagacattactgtggagtggcagtggaatgggcagccagcggagaactacaagaacactcagcccatcatggacacagatggctcttacttcgtctacagcaagctcaatgtgcagaagagcaactgggaggcaggaaatactttcacctgctctgtgttacatgagggcctgcacaaccaccatactgagaagagcctctcccactctcctggtaaatga

SEQ ID NO: 17 - DNA, 1341 bp, Artificial Sequence
  anti-ID heavy chain
caggtccaactgcaacaacctgggtctgagctggtgaggcctggaggttcagtgaagctgtcctgcaaggcttctgactacactttcaccagctactggatgcactgggtgaggcagaggcctggacaaggccttgagtggattggaaatatttatcctggtagtggtggtactaactacgatgagaagttcaagaggaaggccacactgactgtagacacatcctccagcacagcctacatgcagctccgcagcctgacatctgaggactctgcggtctattactgtacaagagaggttactacagtagcttattactattctatggactactggggtcaaggaacctcagtcaccgtctcctcagccaaaacgacacccccatctgtctatccactggcccctggatctgctgcccaaactaactccatggtgaccctgggatgcctggtcaagggctatttccctgagccagtgacagtgacctggaactctggatccctgtccagcggtgtgcacaccttcccagctgtcctgcagtctgacctctacactctgagcagctcagtgactgtcccctccagcacctggcccagcgagaccgtcacctgcaacgttgcccacccggccagcagcaccaaggtggacaagaaaattgtgcccagggattgtggttgtaagccttgcatatgtacagtcccagaagtatcatctgtcttcatcttccccccaaagcccaaggatgtgctcaccattactctgactcctaaggtcacgtgtgttgtggtagacatcagcaaggatgatcccgaggtccagttcagctggtttgtagatgatgtggaggtgcacacagctcagacgcaaccccgggaggagcagttcaacagcactttccgctcagtcagtgaacttcccatcatgcaccaggactggctcaatggcaaggagttcaaatgcagggtcaacagtgcagctttccctgcccccatcgagaaaaccatctccaaaaccaaaggcagaccgaaggctccacaggtgtacaccattccacctcccaaggagcagatggccaaggataaagtcagtctgacctgcatgataacagacttcttccctgaagacattactgtggagtggcagtggaatgggcagccagcggagaactacaagaacactcagcccatcatggacacagatggctcttacttcgtctacagcaagctcaatgtgcagaagagcaactgggaggcaggaaatactttcacctgctctgtgttacatgagggcctgcacaaccaccatactgagaagagcctctcccactctcctggtaaatga

SEQ ID NO: 18 - DNA, 57 bp, Artificial Sequence
  anti-ID HC signal sequence
atgggatggagctctatcatcctcttcttggtagcaacagcctcaggtgtccactcc

SEQ ID NO: 19 - DNA, 321 bp, Artificial Sequence
  anti-ID VL
gatatccagatgacacagactacatcctccctgtctgcctctctgggagacagagtcaccatcagttgcagggcaagtcaggacattagcaattatttaaactggtatcagcagaaaccagatggaactgttaaactcctgatctactacacatcaagattacactcaggagtcccatcaaggttcagtggcagtgggtctggaacagattattctctcaccattagcaacctggagcaagaagatattgccacttacttttgtcagcagggtaaaacggttccattcacgttcggctcggggacaaagttggaaataaaa

SEQ ID NO: 20 - DNA, 324 bp, Artificial Sequence
  anti-ID CL
cgggctgatgctgcaccaactgtatccatcttcccaccatccagtgagcagttaacatctggaggtgcctcagtcgtgtgcttcttgaacaacttctaccccaaagacatcaatgtcaagtggaagattgatggcagtgaacgacaaaatggcgtcctgaacagttggactgatcaggacagcaaagacagcacctacagcatgagcagcaccctcacgttgaccaaggacgagtatgaacgacataacaactatacctgtgaggccactcacaagacatcaacttcacccattgtcaagagcttcaacaggaatgagtgttag

SEQ ID NO: 21 - DNA, 645 bp, Artificial Sequence
  anti-ID light chain
gatatccagatgacacagactacatcctccctgtctgcctctctgggagacagagtcaccatcagttgcagggcaagtcaggacattagcaattatttaaactggtatcagcagaaaccagatggaactgttaaactcctgatctactacacatcaagattacactcaggagtcccatcaaggttcagtggcagtgggtctggaacagattattctctcaccattagcaacctggagcaagaagatattgccacttacttttgtcagcagggtaaaacggttccattcacgttcggctcggggacaaagttggaaataaaacgggctgatgctgcaccaactgtatccatcttcccaccatccagtgagcagttaacatctggaggtgcctcagtcgtgtgcttcttgaacaacttctaccccaaagacatcaatgtcaagtggaagattgatggcagtgaacgacaaaatggcgtcctgaacagttggactgatcaggacagcaaagacagcacctacagcatgagcagcaccctcacgttgaccaaggacgagtatgaacgacataacaactatacctgtgaggccactcacaagacatcaacttcacccattgtcaagagcttcaacaggaatgagtgttag

SEQ ID NO: 22 - DNA, 60 bp, Artificial Sequence
  anti-ID LC signal sequence
atgatgtcctctgctcagttccttggtctcctgttgctctgttttcaaggtaccagatgt

SEQ ID NO: 23 - protein, 122 aa, Mus musculus
  SJ25C1 VH
EVKLQQSGAELVRPGSSVKISCKASGYAFSSYWMNWVKQRPGQGLEWIGQIYPGDGDTNYNGKFKGQATLTADKSSSTAYMQLSGLTSEDSAVYFCARKTISSVVDFYFDYWGQGTTVTVSS

SEQ ID NO: 24 - protein, 108 aa, Mus musculus
  SJ25C1 VL
DIELTQSPKFMSTSVGDRVSVTCKASQNVGTNVAWYQQKPGQSPKPLIYSATYRNSGVPDRFTGSGSGTDFTLTITNVQSKDLADYFCQQYNRYPYTSGGGTKLEIKR

SEQ ID NO: 25 - protein, 15 aa, Artificial Sequence
  Linker
GGGGSGGGGSGGGGS

SEQ ID NO: 26 - protein, 5 aa, Artificial Sequence
  4GS linker
GGGGS

SEQ ID NO: 27 - protein, 39 aa, Artificial Sequence
  An extracellular portion of CD28
IEVMYPPPYLDNEKSNGTIIHVKGKHLCPSPLFPGPSKP

SEQ ID NO: 28 - protein, 245 aa, Mus musculus
  SJ25C1 scFv
EVKLQQSGAELVRPGSSVKISCKASGYAFSSYWMNWVKQRPGQGLEWIGQIYPGDGDTNYNGKFKGQATLTADKSSSTAYMQLSGLTSEDSAVYFCARKTISSVVDFYFDYWGQGTTVTVSSGGGGSGGGGSGGGGSDIELTQSPKFMSTSVGDRVSVTCKASQNVGTNVAWYQQKPGQSPKPLIYSATYRNSGVPDRFTGSGSGTDFTLTITNVQSKDLADYFCQQYNRYPYTSGGGTKLEIKR

SEQ ID NO: 29 - protein, 4 aa, Artificial Sequence
  3GS linker
GGGS

SEQ ID NO: 30 - protein, 120 aa, Mus musculus
  FMC63 VH
EVKLQESGPGLVAPSQSLSVTCTVSGVSLPDYGVSWIRQPPRKGLEWLGVIWGSETTYYNSALKSRLTIIKDNSKSQVFLKMNSLQTDDTAIYYCAKHYYYGGSYAMDYWGQGTSVTVSS

SEQ ID NO: 31 - protein, 107 aa, Mus musculus
  FMC63 VL
DIQMTQTTSSLSASLGDRVTISCRASQDISKYLNWYQQKPDGTVKLLIYHTSRLHSGVPSRFSGSGSGTDYSLTISNLEQEDIATYFCQQGNTLPYTFGGGTKLEIT

SEQ ID NO: 32 - protein, 220 aa, Artificial Sequence
  IgG1 Fc lacking hinge
PCPAPELLGGPSVFLFPPKPKDTLMISRTPEVTCVVVDVSHEDPEVKFNWYVDGVEVHNAKTKPREEQYNSTYRVVSVLTVLHQDWLNGKEYKCKVSNKALPAPIEKTISKAKGQPREPQVYTLPPSREEMTKNQVSLTCLVKGFYPSDIAVEWESNGQPENNYKTTPPVLDSDGSFFLYSKLTVDKSRWQQGNVFSCSVMHEALHNHYTQKSLSLSPGK

SEQ ID NO: 33 - protein, 18 aa, Artificial Sequence
  Linker
GSTSGSGKPGSGEGSTKG

SEQ ID NO: 34 - protein, 245 aa, Artificial Sequence
  FMC63 scFv
DIQMTQTTSSLSASLGDRVTISCRASQDISKYLNWYQQKPDGTVKLLIYHTSRLHSGVPSRFSGSGSGTDYSLTISNLEQEDIATYFCQQGNTLPYTFGGGTKLEITGSTSGSGKPGSGEGSTKGEVKLQESGPGLVAPSQSLSVTCTVSGVSLPDYGVSWIRQPPRKGLEWLGVIWGSETTYYNSALKSRLTIIKDNSKSQVFLKMNSLQTDDTAIYYCAKHYYYGGSYAMDYWGQGTSVTVSS

SEQ ID NO: 35 - protein, 465 aa, Artificial Sequence
  FMC63 reagent
DIQMTQTTSSLSASLGDRVTISCRASQDISKYLNWYQQKPDGTVKLLIYHTSRLHSGVPSRFSGSGSGTDYSLTISNLEQEDIATYFCQQGNTLPYTFGGGTKLEITGSTSGSGKPGSGEGSTKGEVKLQESGPGLVAPSQSLSVTCTVSGVSLPDYGVSWIRQPPRKGLEWLGVIWGSETTYYNSALKSRLTIIKDNSKSQVFLKMNSLQTDDTAIYYCAKHYYYGGSYAMDYWGQGTSVTVSSPCPAPELLGGPSVFLFPPKPKDTLMISRTPEVTCVVVDVSHEDPEVKFNWYVDGVEVHNAKTKPREEQYNSTYRVVSVLTVLHQDWLNGKEYKCKVSNKALPAPIEKTISKAKGQPREPQVYTLPPSREEMTKNQVSLTCLVKGFYPSDIAVEWESNGQPENNYKTTPPVLDSDGSFFLYSKLTVDKSRWQQGNVFSCSVMHEALHNHYTQKSLSLSPGK

SEQ ID NO: 36 - protein, 122 aa, Artificial Sequence
  anti-ID B-1 VH
EVQLQQSGPELVKPGASVKMSCKASGYTFTDYYMKWVKQCHGKSLEWIGDINPNNGGTDYNQNFKGKATLTVDKSSSTAYMQLNSLTSEDSAVYYCAREGNNYGSRDAMDYWGQGTSVTVSS

SEQ ID NO: 37 - protein, 330 aa, Artificial Sequence
  anti-ID B-1 CH
AKTTAPSVYPLAPVCGDTTGSSVTLGCLVKGYFPEPVTLTWNSGSLSSGVHTFPAVLQSDLYTLSSSVTVTSSTWPSQSITCNVAHPASSTKVDKKIEPRGPTIKPCPPCKCPAPNLLGGPSVFIFPPKIKDVLMISLSPIVTCVVVDVSEDDPDVQISWFVNNVEVHTAQTQTHREDYNSTLRVVSALPIQHQDWMSGKEFKCKVNNKDLPAPIERTISKPKGSVRAPQVYVLPPPEEEMTKKQVTLTCMVTDFMPEDIYVEWTNNGKTELNYKNTEPVLDSDGSYFMYSKLRVEKKNWVERNSYSCSVVHEGLHNHHTTKSFSRTPGK

SEQ ID NO: 38 - protein, 452 aa, Artificial Sequence
  anti-ID B-1 heavy chain
EVQLQQSGPELVKPGASVKMSCKASGYTFTDYYMKWVKQCHGKSLEWIGDINPNNGGTDYNQNFKGKATLTVDKSSSTAYMQLNSLTSEDSAVYYCAREGNNYGSRDAMDYWGQGTSVTVSSAKTTAPSVYPLAPVCGDTTGSSVTLGCLVKGYFPEPVTLTWNSGSLSSGVHTFPAVLQSDLYTLSSSVTVTSSTWPSQSITCNVAHPASSTKVDKKIEPRGPTIKPCPPCKCPAPNLLGGPSVFIFPPKIKDVLMISLSPIVTCVVVDVSEDDPDVQISWFVNNVEVHTAQTQTHREDYNSTLRVVSALPIQHQDWMSGKEFKCKVNNKDLPAPIERTISKPKGSVRAPQVYVLPPPEEEMTKKQVTLTCMVTDFMPEDIYVEWTNNGKTELNYKNTEPVLDSDGSYFMYSKLRVEKKNWVERNSYSCSVVHEGLHNHHTTKSFSRTPGK

SEQ ID NO: 39 - protein, 19 aa, Artificial Sequence
  anti-ID B-1 HC signal sequence
MGWSWIFLFLLSGTAGVLS

SEQ ID NO: 40 - protein, 106 aa, Artificial Sequence
  anti-ID B-1 VL
QIVLTQSPALMSASPGEKVTMTCSASSGVIYMYWYQQKPRSSPKPWIYLTSNLASGVPARFSGSGSGTSYSLTISSMEAEDAATYYCQQWSSNPLTFGAGTKLELK

SEQ ID NO: 41 - protein, 107 aa, Artificial Sequence
  anti-ID B-1 CL
RADAAPTVSIFPPSSEQLTSGGASVVCFLNNFYPKDINVKWKIDGSERQNGVLNSWTDQDSKDSTYSMSSTLTLTKDEYERHNSYTCEATHKTSTSPIVKSFNRNEC

SEQ ID NO: 42 - protein, 213 aa, Artificial Sequence
  anti-ID B-1 light chain
QIVLTQSPALMSASPGEKVTMTCSASSGVIYMYWYQQKPRSSPKPWIYLTSNLASGVPARFSGSGSGTSYSLTISSMEAEDAATYYCQQWSSNPLTFGAGTKLELKRADAAPTVSIFPPSSEQLTSGGASVVCFLNNFYPKDINVKWKIDGSERQNGVLNSWTDQDSKDSTYSMSSTLTLTKDEYERHNSYTCEATHKTSTSPIVKSFNRNEC

SEQ ID NO: 43 - protein, 22 aa, Artificial Sequence
  anti-ID B-1 LC signal sequence
MDFQVQIFSFLLMSASVIMSRG

SEQ ID NO: 44 - protein, 5 aa, Artificial Sequence
  anti-ID B-1 HC-CDR1
DYYMK

SEQ ID NO: 45 - protein, 17 aa, Artificial Sequence
  anti-ID B-1 HC-CDR2
DINPNNGGTDYNQNFKG

SEQ ID NO: 46 - protein, 13 aa, Artificial Sequence
  anti-ID B-1 HC-CDR3
EGNNYGSRDAMDY

SEQ ID NO: 47 - protein, 10 aa, Artificial Sequence
  anti-ID B-1 LC-CDR1
SASSGVIYMY

SEQ ID NO: 48 - protein, 7 aa, Artificial Sequence
  anti-ID B-1 LC-CDR2
LTSNLAS

SEQ ID NO: 49 - protein, 9 aa, Artificial Sequence
  anti-ID B-1 LC-CDR3
QQWSSNPLT

SEQ ID NO: 50 - DNA, 366 bp, Artificial Sequence
  anti-ID B-1 VH
gaggtccagctgcaacaatctggacctgagctggtgaagcctggggcttcagtgaagatgtcctgtaaggcttctggatacacattcactgactactacatgaagtgggtgaagcagtgtcatggaaagagccttgagtggattggagatattaatcctaacaatggtggtactgactacaaccagaactttaagggcaaggccacattgactgtagacaaatcctccagcacagcctacatgcagctcaacagcctgacatctgaggactctgcagtctattactgtgcaagagaggggaataactacggtagtagagatgctatggactactggggtcaaggaacgtcagtcaccgtctcctca

SEQ ID NO: 51 - DNA, 990 bp, Artificial Sequence
  anti-ID B-1 CH
gccaaaacaacagccccatcggtctatccactggcccctgtgtgtggagatacaactggctcctcggtgactctaggatgcctggtcaagggttatttccctgagccagtgaccttgacctggaactctggatccctgtccagtggtgtgcacaccttcccagctgtcctgcagtctgacctctacaccctcagcagctcagtgactgtaacctcgagcacctggcccagccagtccatcacctgcaatgtggcccacccggcaagcagcaccaaggtggacaagaaaattgagcccagagggcccacaatcaagccctgtcctccatgcaaatgcccagcacctaacctcttgggtggaccatccgtcttcatcttccctccaaagatcaaggatgtactcatgatctccctgagccccatagtcacatgtgtggtggtggatgtgagcgaggatgacccagatgtccagatcagctggtttgtgaacaacgtggaagtacacacagctcagacacaaacccatagagaggattacaacagtactctccgggtggtcagtgccctccccatccagcaccaggactggatgagtggcaaggagttcaaatgcaaggtcaacaacaaagacctcccagcgcccatcgagagaaccatctcaaaacccaaagggtcagtaagagctccacaggtatatgtcttgcctccaccagaagaagagatgactaagaaacaggtcactctgacctgcatggtcacagacttcatgcctgaagacatttacgtggagtggaccaacaacgggaaaacagagctaaactacaagaacactgaaccagtcctggactctgatggttcttacttcatgtacagcaagctgagagtggaaaagaagaactgggtggaaagaaatagctactcctgttcagtggtccacgagggtctgcacaatcaccacacgactaagagcttctcccggactccgggtaaa

SEQ ID NO: 52 - DNA, 1356 bp, Artificial Sequence
  anti-ID B-1 heavy chain
gaggtccagctgcaacaatctggacctgagctggtgaagcctggggcttcagtgaagatgtcctgtaaggcttctggatacacattcactgactactacatgaagtgggtgaagcagtgtcatggaaagagccttgagtggattggagatattaatcctaacaatggtggtactgactacaaccagaactttaagggcaaggccacattgactgtagacaaatcctccagcacagcctacatgcagctcaacagcctgacatctgaggactctgcagtctattactgtgcaagagaggggaataactacggtagtagagatgctatggactactggggtcaaggaacgtcagtcaccgtctcctcagccaaaacaacagccccatcggtctatccactggcccctgtgtgtggagatacaactggctcctcggtgactctaggatgcctggtcaagggttatttccctgagccagtgaccttgacctggaactctggatccctgtccagtggtgtgcacaccttcccagctgtcctgcagtctgacctctacaccctcagcagctcagtgactgtaacctcgagcacctggcccagccagtccatcacctgcaatgtggcccacccggcaagcagcaccaaggtggacaagaaaattgagcccagagggcccacaatcaagccctgtcctccatgcaaatgcccagcacctaacctcttgggtggaccatccgtcttcatcttccctccaaagatcaaggatgtactcatgatctccctgagccccatagtcacatgtgtggtggtggatgtgagcgaggatgacccagatgtccagatcagctggtttgtgaacaacgtggaagtacacacagctcagacacaaacccatagagaggattacaacagtactctccgggtggtcagtgccctccccatccagcaccaggactggatgagtggcaaggagttcaaatgcaaggtcaacaacaaagacctcccagcgcccatcgagagaaccatctcaaaacccaaagggtcagtaagagctccacaggtatatgtcttgcctccaccagaagaagagatgactaagaaacaggtcactctgacctgcatggtcacagacttcatgcctgaagacatttacgtggagtggaccaacaacgggaaaacagagctaaactacaagaacactgaaccagtcctggactctgatggttcttacttcatgtacagcaagctgagagtggaaaagaagaactgggtggaaagaaatagctactcctgttcagtggtccacgagggtctgcacaatcaccacacgactaagagcttctcccggactccgggtaaa

SEQ ID NO: 53 - DNA, 57 bp, Artificial Sequence
  anti-ID B-1 HC signal sequence
atgggatggagctggatctttctcttcctcttgtcaggaactgcaggtgtcctctct

SEQ ID NO: 54 - DNA, 318 bp, Artificial Sequence
  anti-ID B-1 VL
caaattgttctcacccagtctccagcactcatgtctgcatctccaggggagaaggtcaccatgacctgcagtgccagctcaggtgtaatttacatgtactggtaccaacagaagccaagatcctcccccaaaccctggatttatctcacatccaacctggcttctggagtccctgctcgcttcagtggcagtgggtctgggacctcttactctctcacaatcagcagcatggaggctgaagatgctgccacttattactgccagcagtggagtagtaacccgctcacgttcggtgctggcaccaagctggagctgaaa

SEQ ID NO: 55 - DNA, 321 bp, Artificial Sequence
  anti-ID B-1 CL
cgggctgatgctgcaccaactgtatccatcttcccaccatccagtgagcagttaacatctggaggtgcctcagtcgtgtgcttcttgaacaacttctaccccaaagacatcaatgtcaagtggaagattgatggcagtgaacgacaaaatggcgtcctgaacagttggactgatcaggacagcaaagacagcacctacagcatgagcagcaccctcacgttgaccaaggacgagtatgaacgacataacagctatacctgtgaggccactcacaagacatcaacttcacccattgtcaagagcttcaacaggaatgagtgt

SEQ ID NO: 56 - DNA, 639 bp, Artificial Sequence
  anti-ID B-1 light chain
caaattgttctcacccagtctccagcactcatgtctgcatctccaggggagaaggtcaccatgacctgcagtgccagctcaggtgtaatttacatgtactggtaccaacagaagccaagatcctcccccaaaccctggatttatctcacatccaacctggcttctggagtccctgctcgcttcagtggcagtgggtctgggacctcttactctctcacaatcagcagcatggaggctgaagatgctgccacttattactgccagcagtggagtagtaacccgctcacgttcggtgctggcaccaagctggagctgaaacgggctgatgctgcaccaactgtatccatcttcccaccatccagtgagcagttaacatctggaggtgcctcagtcgtgtgcttcttgaacaacttctaccccaaagacatcaatgtcaagtggaagattgatggcagtgaacgacaaaatggcgtcctgaacagttggactgatcaggacagcaaagacagcacctacagcatgagcagcaccctcacgttgaccaaggacgagtatgaacgacataacagctatacctgtgaggccactcacaagacatcaacttcacccattgtcaagagcttcaacaggaatgagtgt

SEQ ID NO: 57 - DNA, 66 bp, Artificial Sequence
  anti-ID B-1 LC signal sequence
atggattttcaagtgcagattttcagcttcctgctaatgagtgcctcagtcataatgtccagggga

SEQ ID NO: 58 - protein, 115 aa, Artificial Sequence
  anti-ID B-2 VH
QVQLQQPGAELVRPGASVKLSCKTSGYSFTRYWMNWVKQRPGQGLEWIGMIHPSDSETRLNQKFKDKATLTVDNSSSTAYMQLSSPTSEDSAVYYCASIYYEEAWGQGTLVTVSA

SEQ ID NO: 59 - protein, 324 aa, Artificial Sequence; identical to SEQ ID NO: 2
  anti-ID B-2 CH

SEQ ID NO: 60 - protein, 439 aa, Artificial Sequence
  anti-ID B-2 heavy chain
QVQLQQPGAELVRPGASVKLSCKTSGYSFTRYWMNWVKQRPGQGLEWIGMIHPSDSETRLNQKFKDKATLTVDNSSSTAYMQLSSPTSEDSAVYYCASIYYEEAWGQGTLVTVSAAKTTPPSVYPLAPGSAAQTNSMVTLGCLVKGYFPEPVTVTWNSGSLSSGVHTFPAVLQSDLYTLSSSVTVPSSTWPSETVTCNVAHPASSTKVDKKIVPRDCGCKPCICTVPEVSSVFIFPPKPKDVLTITLTPKVTCVVVDISKDDPEVQFSWFVDDVEVHTAQTQPREEQFNSTFRSVSELPIMHQDWLNGKEFKCRVNSAAFPAPIEKTISKTKGRPKAPQVYTIPPPKEQMAKDKVSLTCMITDFFPEDITVEWQWNGQPAENYKNTQPIMDTDGSYFVYSKLNVQKSNWEAGNTFTCSVLHEGLHNHHTEKSLSHSPGK

SEQ ID NO: 61 - protein, 19 aa, Artificial Sequence
  anti-ID B-2 HC signal sequence
MGWSSIILFLVATATGVHS

SEQ ID NO: 62 - protein, 107 aa, Artificial Sequence
  anti-ID B-2 VL
DIQMTQSPASLSASVGETVTITCRASGNIHNYLAWYQQKQGKSPQLLVYNAKTLADSVPSRFSGSGSGTQYSLKINSLQPEDFGSYYCQHFWSTPYTFGGGTKLEIK

SEQ ID NO: 63 - protein, 214 aa, Artificial Sequence
  anti-ID B-2 light chain
DIQMTQSPASLSASVGETVTITCRASGNIHNYLAWYQQKQGKSPQLLVYNAKTLADSVPSRFSGSGSGTQYSLKINSLQPEDFGSYYCQHFWSTPYTFGGGTKLEIKRADAAPTVSIFPPSSEQLTSGGASVVCFLNNFYPKDINVKWKIDGSERQNGVLNSWTDQDSKDSTYSMSSTLTLTKDEYERHNSYTCEATHKTSTSPIVKSFNRNEC

SEQ ID NO: 64 - protein, 20 aa, Artificial Sequence
  anti-ID B-2 LC signal sequence
MSVLTQVLALLLLWLTGARC

SEQ ID NO: 65 - protein, 5 aa, Artificial Sequence
  anti-ID B-2 HC-CDR1
RYWMN

SEQ ID NO: 66 - protein, 17 aa, Artificial Sequence
  anti-ID B-2 HC-CDR2
MIHPSDSETRLNQKFKD

SEQ ID NO: 67 - protein, 6 aa, Artificial Sequence
  anti-ID B-2 HC-CDR3
IYYEEA

SEQ ID NO: 68 - protein, 11 aa, Artificial Sequence
  anti-ID B-2 LC-CDR1
RASGNIHNYLA

SEQ ID NO: 69 - protein, 7 aa, Artificial Sequence
  anti-ID B-2 LC-CDR2
NAKTLAD

SEQ ID NO: 70 - protein, 9 aa, Artificial Sequence
  anti-ID B-2 LC-CDR3
QHFWSTPYT

SEQ ID NO: 71 - DNA, 345 bp, Artificial Sequence
  anti-ID B-2 VH
caggtccaactgcagcagcctggggctgagctggtgaggcctggagcttcagtgaagctgtcctgcaagacttctggctactccttcaccaggtactggatgaactgggtgaagcagaggcctggacaaggccttgagtggattggcatgattcatccttccgatagtgaaactaggttaaatcagaagttcaaggacaaggccacattgactgtagacaattcctccagcacagcctacatgcaactcagcagcccgacatctgaggactctgcggtctattactgtgcaagcatctactatgaagaggcctggggccaagggactctggtcactgtctctgca

SEQ ID NO: 72 - DNA, 972 bp, Artificial Sequence
  anti-ID B-2 CH
gccaaaacgacacccccatctgtctatccactggcccctggatctgctgcccaaactaactccatggtgaccctgggatgcctggtcaagggctatttccctgagccagtgacagtgacctggaactctggatccctgtccagcggtgtgcacaccttcccagctgtcctgcagtctgacctctacactctgagcagctcagtgactgtcccctccagcacctggcccagcgagaccgtcacctgcaacgttgcccacccggccagcagcaccaaggtggacaagaaaattgtgcccagggattgtggttgtaagccttgcatatgtacagtcccagaagtatcatctgtcttcatcttccccccaaagcccaaggatgtgctcaccattactctgactcctaaggtcacgtgtgttgtggtagacatcagcaaggatgatcccgaggtccagttcagctggtttgtagatgatgtggaggtgcacacagctcagacgcaaccccgggaggagcagttcaacagcactttccgctcagtcagtgaacttcccatcatgcaccaggactggctcaatggcaaggagttcaaatgcagggtcaacagtgcagctttccctgcccccatcgagaaaaccatctccaaaaccaaaggcagaccgaaggctccacaggtgtacaccattccacctcccaaggagcagatggccaaggataaagtcagtctgacctgcatgataacagacttcttccctgaagacattactgtggagtggcagtggaatgggcagccagcggagaactacaagaacactcagcccatcatggacacagatggctcttacttcgtctacagcaagctcaatgtgcagaagagcaactgggaggcaggaaatactttcacctgctctgtgttacatgagggcctgcacaaccaccatactgagaagagcctctcccactctcctggtaaa

SEQ ID NO: 73 - DNA, 1317 bp, Artificial Sequence
  anti-ID B-2 heavy chain
caggtccaactgcagcagcctggggctgagctggtgaggcctggagcttcagtgaagctgtcctgcaagacttctggctactccttcaccaggtactggatgaactgggtgaagcagaggcctggacaaggccttgagtggattggcatgattcatccttccgatagtgaaactaggttaaatcagaagttcaaggacaaggccacattgactgtagacaattcctccagcacagcctacatgcaactcagcagcccgacatctgaggactctgcggtctattactgtgcaagcatctactatgaagaggcctggggccaagggactctggtcactgtctctgcagccaaaacgacacccccatctgtctatccactggcccctggatctgctgcccaaactaactccatggtgaccctgggatgcctggtcaagggctatttccctgagccagtgacagtgacctggaactctggatccctgtccagcggtgtgcacaccttcccagctgtcctgcagtctgacctctacactctgagcagctcagtgactgtcccctccagcacctggcccagcgagaccgtcacctgcaacgttgcccacccggccagcagcaccaaggtggacaagaaaattgtgcccagggattgtggttgtaagccttgcatatgtacagtcccagaagtatcatctgtcttcatcttccccccaaagcccaaggatgtgctcaccattactctgactcctaaggtcacgtgtgttgtggtagacatcagcaaggatgatcccgaggtccagttcagctggtttgtagatgatgtggaggtgcacacagctcagacgcaaccccgggaggagcagttcaacagcactttccgctcagtcagtgaacttcccatcatgcaccaggactggctcaatggcaaggagttcaaatgcagggtcaacagtgcagctttccctgcccccatcgagaaaaccatctccaaaaccaaaggcagaccgaaggctccacaggtgtacaccattccacctcccaaggagcagatggccaaggataaagtcagtctgacctgcatgataacagacttcttccctgaagacattactgtggagtggcagtggaatgggcagccagcggagaactacaagaacactcagcccatcatggacacagatggctcttacttcgtctacagcaagctcaatgtgcagaagagcaactgggaggcaggaaatactttcacctgctctgtgttacatgagggcctgcacaaccaccatactgagaagagcctctcccactctcctggtaaa

SEQ ID NO: 74 - DNA, 57 bp, Artificial Sequence
  anti-ID B-2 HC signal sequence
atgggatggagctctatcatcctcttcttggtagcaacagctacaggtgtccactcc

SEQ ID NO: 75 - DNA, 321 bp, Artificial Sequence
  anti-ID B-2 VL
gacatccagatgactcagtctccagcctccctatctgcatctgtgggagaaactgtcaccatcacatgtcgagcaagtgggaatattcacaattatttagcatggtatcagcagaaacagggaaaatctcctcagctcctggtctataatgcaaaaaccttagcagatagtgtgccatcaaggttcagtggcagtggatcaggaacacaatattctctcaagatcaacagcctgcagcctgaagattttgggagttattactgtcaacatttttggagtactccgtacacgttcggaggggggaccaagctggaaataaaa

SEQ ID NO: 76 - DNA, 642 bp, Artificial Sequence
  anti-ID B-2 light chain
gacatccagatgactcagtctccagcctccctatctgcatctgtgggagaaactgtcaccatcacatgtcgagcaagtgggaatattcacaattatttagcatggtatcagcagaaacagggaaaatctcctcagctcctggtctataatgcaaaaaccttagcagatagtgtgccatcaaggttcagtggcagtggatcaggaacacaatattctctcaagatcaacagcctgcagcctgaagattttgggagttattactgtcaacatttttggagtactccgtacacgttcggaggggggaccaagctggaaataaaacgggctgatgctgcaccaactgtatccatcttcccaccatccagtgagcagttaacatctggaggtgcctcagtcgtgtgcttcttgaacaacttctaccccaaagacatcaatgtcaagtggaagattgatggcagtgaacgacaaaatggcgtcctgaacagttggactgatcaggacagcaaagacagcacctacagcatgagcagcaccctcacgttgaccaaggacgagtatgaacgacataacagctatacctgtgaggccactcacaagacatcaacttcacccattgtcaagagcttcaacaggaatgagtgt

SEQ ID NO: 77 - DNA, 60 bp, Artificial Sequence
  anti-ID B-2 LC signal sequence
atgagtgtgctcactcaggtcctggcgttgctgctgctgtggcttacaggtgccagatgt

SEQ ID NO: 78 - protein, 7 aa, Artificial Sequence
  anti-ID HC-CDR1
DYTFTSY

SEQ ID NO: 79 - protein, 10 aa, Artificial Sequence
  anti-ID HC-CDR1
DYTFTSYWMH

SEQ ID NO: 80 - protein, 6 aa, Artificial Sequence
  anti-ID HC-CDR1
TSYWMH

SEQ ID NO: 81 - protein, 6 aa, Artificial Sequence
  anti-ID HC-CDR2
YPGSGG

SEQ ID NO: 82 - protein, 10 aa, Artificial Sequence
  anti-ID HC-CDR2
NIYPGSGGTN

SEQ ID NO: 83 - protein, 13 aa, Artificial Sequence
  anti-ID HC-CDR2
WIGNIYPGSGGTN

SEQ ID NO: 84 - protein, 14 aa, Artificial Sequence
  anti-ID HC-CDR3
TREVTTVAYYYSMD

SEQ ID NO: 85 - protein, 7 aa, Artificial Sequence
  anti-ID LC-CDR1
SNYLNWY

SEQ ID NO: 86 - protein, 10 aa, Artificial Sequence
  anti-ID LC-CDR2
LLIYYTSRLH

SEQ ID NO: 87 - protein, 8 aa, Artificial Sequence
  anti-ID LC-CDR3
QQGKTVPF

SEQ ID NO: 88 - protein, 7 aa, anti-ID B-1 HC-CDR1
GYTFTDY

SEQ ID NO: 89 - protein, 10 aa, Artificial Sequence
  anti-ID B-1 HC-CDR1
GYTFTDYYMK

SEQ ID NO: 90 - protein, 6 aa, Artificial Sequence
  anti-ID B-1 HC-CDR1
TDYYMK

SEQ ID NO: 91 - protein, 6 aa, Artificial Sequence
  anti-ID B-1 HC-CDR2
NPNNGG

SEQ ID NO: 92 - protein, 10 aa, Artificial Sequence
  anti-ID B-1 HC-CDR2
DINPNNGGTD

SEQ ID NO: 93 - protein, 13 aa, Artificial Sequence
  anti-ID B-1 HC-CDR2
WIGDINPNNGGTD

SEQ ID NO: 94 - protein, 14 aa, Artificial Sequence
  anti-ID B-1 HC-CDR3
AREGNNYGSRDAMD

SEQ ID NO: 95 - protein, 6 aa, Artificial Sequence
  anti-ID B-1 LC-CDR1
IYMYWY

SEQ ID NO: 96 - protein, 10 aa, Artificial Sequence
  anti-ID B-1 LC-CDR2
PWIYLTSNLA

SEQ ID NO: 97 - protein, 8 aa, Artificial Sequence
  anti-ID B-1 LC-CDR3
QQWSSNPL

SEQ ID NO: 98 - protein, 7 aa, Artificial Sequence
  anti-ID B-2 HC-CDR1
GYSFTRY

SEQ ID NO: 99 - protein, 10 aa, Artificial Sequence
  anti-ID B-2 HC-CDR1
GYSFTRYWMN

SEQ ID NO: 100 - protein, 6 aa, Artificial Sequence
  anti-ID B-2 HC-CDR1
TRYWMN

SEQ ID NO: 101 - protein, 6 aa, Artificial Sequence
  anti-ID B-2 HC-CDR2
HPSDSE

SEQ ID NO: 102 - protein, 10 aa, Artificial Sequence
  anti-ID B-2 HC-CDR2
MIHPSDSETR

SEQ ID NO: 103 - protein, 13 aa, Artificial Sequence
  anti-ID B-2 HC-CDR2
WIGMIHPSDSETR

SEQ ID NO: 104 - protein, 7 aa, Artificial Sequence
  anti-ID B-2 HC-CDR3
ASIYYEE

SEQ ID NO: 105 - protein, 7 aa, Artificial Sequence
  anti-ID B-2 LC-CDR1
HNYLAWY

SEQ ID NO: 106 - protein, 10 aa, Artificial Sequence
  anti-ID B-2 LC-CDR2
LLVYNAKTLA

SEQ ID NO: 107 - protein, 8 aa, Artificial Sequence
  anti-ID B-2 LC-CDR3
QHFWSTPY

SEQ ID NO: 108 - protein, 10 aa, Artificial Sequence
  HC-CDR1 Consensus
  VARIANT 3: Xaa = T or S
  VARIANT 5: Xaa = T or S
  VARIANT 6: Xaa = D or R
  VARIANT 8: Xaa = Y or W
  VARIANT 10: Xaa = K or N
GYXFXXYXMX

SEQ ID NO: 109 - protein, 20 aa, Artificial Sequence
  HC-CDR2 Consensus
  VARIANT 4: Xaa = D or M
  VARIANT 6: Xaa = N or H
  VARIANT 8: Xaa = N or S
  VARIANT 9: Xaa = N or D
  VARIANT 10: Xaa = G or S
  VARIANT (11)...(11): Xaa = G or E
  VARIANT (13)...(13): Xaa = D or R
  VARIANT (14)...(14): Xaa = Y or L
  VARIANT (17)...(17): Xaa = N or K
  VARIANT (20)...(20): Xaa = G or D
WIGXIXPXXXXTXXNQXFKX

SEQ ID NO: 110 - protein, 15 aa, Artificial Sequence
  HC-CDR3 Consensus
  VARIANT 2: Xaa = R or S
  VARIANT 3: Xaa = E or I
  VARIANT 4: Xaa = G or Y
  VARIANT 5: Xaa = N or Y
  VARIANT 6: Xaa = N or E
  VARIANT (7)...(7): Xaa = Y or nul
  VARIANT (8)...(8): Xaa = G or null
  VARIANT (9)...(9): Xaa = S or null
  VARIANT (10)...(10): Xaa = R or null
  VARIANT (11)...(11): Xaa = D or null
  VARIANT (12)...(12): Xaa = A or null
  VARIANT (13)...(13): X13 = M or null
  VARIANT (14)...(14): X14 = D or E
  VARIANT (15)...(15): X15 = Y or A
AXXXXXXXXXXXXXX

SEQ ID NO: 111 - protein, 13 aa, Artificial Sequence
  LC-CDR1 Consensus
  VARIANT (1)...(1): Xaa = S or R
  VARIANT (3)...(3): Xaa = S or R
  VARIANT (4)...(4): Xaa = S or G
  VARIANT (5)...(5): Xaa = G or N
  VARIANT (6)...(6): Xaa = V or I
  VARIANT (7)...(7): Xaa = I or H
  VARIANT (8)...(8): Xaa = N or null
  VARIANT (10)...(10): Xaa = M or L
  VARIANT (11)...(11): Xaa = Y or A
XAXXXXXXYXXWY

SEQ ID NO: 112 - protein, 11 aa, Artificial Sequence
  LC-CDR2 Consensus
  VARIANT (1)...(1): Xaa = P or L
  VARIANT (2)...(2): Xaa = W or L
  VARIANT (3)...(3): Xaa = I or V
  VARIANT (5)...(5): Xaa = L or N
  VARIANT (6)...(6): Xaa = T or A
  VARIANT (7)...(7): Xaa = S or K
  VARIANT (8)...(8): Xaa = N or T
  VARIANT (11)...(11): Xaa = S or D
XXXYXXXXLAX

SEQ ID NO: 113 - protein, 9 aa, Artificial Sequence
  LC-CDR3 Consensus
  VARIANT (2)...(2): Xaa = Q or H
  VARIANT (3)...(3): Xaa =W or F
  VARIANT (4)...(4): Xaa = S or W
  VARIANT (5)...(5): Xaa = S or W
  VARIANT (6)...(6): Xaa = N or T
  VARIANT (8)...(8): Xaa = L or Y
QXXXXXPXT

SEQ ID NO: 114 - protein, 5 aa, Mus musculus
  SJ25C1 HC-CDR1
SYWMN

SEQ ID NO: 115 - protein, 17 aa, Mus musculus
  SJ25C1 HC-CDR2
QIYPGDGDTNYNGKFKG

SEQ ID NO: 116 - protein, 13 aa, Mus musculus
  SJ25C1 HC-CDR3
KTISSVVDFYFDY

SEQ ID NO: 117 - protein, 11 aa, Mus musculus
  SJ25C1 LC-CDR1
KASQNVGTNVA

SEQ ID NO: 118 - protein, 7 aa, Mus musculus
  SJ25C1 LC-CDR2
SATYRNS

SEQ ID NO: 119 - protein, 9 aa, Mus musculus
  SJ25C1 LC-CDR3
QQYNRYPYT

SEQ ID NO: 120 - protein, 5 aa, Mus musculus
  SJ25C1 LC-CDR3
DYGVS

SEQ ID NO: 121 - protein, 16 aa, Mus musculus
  FMC63 HC-CDR2
VIWGSETTYYNSALKS

SEQ ID NO: 122 - protein, 12 aa, Mus musculus
  FMC63 HC-CDR3
HYYYGGSYAMDY

SEQ ID NO: 123 - protein, 11 aa, Mus musculus
  FMC63 LC-CDR1
RASQDISKYLN

SEQ ID NO: 124 - protein, 7 aa, Mus musculus
  FMC63 LC-CDR2
HTSRLHS

SEQ ID NO: 125 - protein, 9 aa, Mus musculus
  FMC63 LC-CDR3
QQGNTLPYT

SEQ ID NO: 126 - protein, 24 aa, Artificial Sequence
  T2A
LEGGGEGRGSLLTCGDVEENPGPR

SEQ ID NO: 127 - protein, 18 aa, Artificial Sequence
  T2A
EGRGSLLTCGDVEENPGP

SEQ ID NO: 128 - protein, 22 aa, Artificial Sequence
  P2A
GSGATNFSLLKQAGDVEENPGP

SEQ ID NO: 129 - protein, 19 aa, Artificial Sequence
  P2A
ATNFSLLKQAGDVEENPGP

SEQ ID NO: 130 - protein, 20 aa, Artificial Sequence
  E2A
QCTNYALLKLAGDVESNPGP

SEQ ID NO: 131 - protein, 22 aa, Artificial Sequence
  F2A
VKQTLNFDLLKLAGDVESNPGP

SEQ ID NO: 132 - protein, 459 aa, Artificial Sequence
  Exemplary humanized anti-SJ25C1 heavy chain
QVQLKQSGPGLVQPSQSLSITCTVSDYTFTSYGVHWVRQSPGKGLEWLGVIYPGSGGTDYNTPFTSRLSINKDNSKSQVFFKMNSLQSNDTAIYYCAREVTTVAYYYSMDYWGQGTLVTVSATLVTVSAASTKGPSVFPLAPSSKSTSGGTAALGCLVKDYFPEPVTVSWNSGALTSGVHTFPAVLQSSGLYSLSSVVTVPSSSLGTQTYICNVNHKPSNTKVDKKVEPKSCDKTHTCPPCPAPELLGGPSVFLFPPKPKDTLMISRTPEVTCVVVDVSHEDPEVKFNWYVDGVEVHNAKTKPREEQYNSTYRVVSVLTVLHQDWLNGKEYKCKVSNKALPAPIEKTISKAKGQPREPQVYTLPPSRDELTKNQVSLTCLVKGFYPSDIAVEWESNGQPENNYKTTPPVLDSDGSFFLYSKLTVDKSRWQQGNVFSCSVMHEALHNHYTQKSLSLSPGK

SEQ ID NO: 133 - protein, 214 aa, Artificial Sequence
  Exemplary humanized anti-SJ25C1 light chain
DILLTQSPVILSVSPGERVSFSCRASQDISNYLNWYQQRTNGSPRLLIKYTSRLHSGIPSRFSGSGSGTDFTLSINSVESEDIADYYCQQGKTVPFTFGAGTKLELKRTVAAPSVFIFPPSDEQLKSGTASVVCLLNNFYPREAKVQWKVDNALQSGNSQESVTEQDSKDSTYSLSSTLTLSKADYEKHKVYACEVTHQGLSSPVTKSFNRGEC

SEQ ID NO: 134 - protein, 459 aa, Artificial Sequence
  Exemplary humanized anti-SJ25C1 heavy chain
QVQLKQSGPGLVQPSQSLSITCTVSGFSLTSYWMHWVRQSPGKGLEWIGNIYPGSGGTNYNTPFTSRLSINKDNSKSQVFFKMNSLQSNDTAIYYCTREVTTVAYYYSMDYWGQGTLVTVSATLVTVSAASTKGPSVFPLAPSSKSTSGGTAALGCLVKDYFPEPVTVSWNSGALTSGVHTFPAVLQSSGLYSLSSVVTVPSSSLGTQTYICNVNHKPSNTKVDKKVEPKSCDKTHTCPPCPAPELLGGPSVFLFPPKPKDTLMISRTPEVTCVVVDVSHEDPEVKFNWYVDGVEVHNAKTKPREEQYNSTYRVVSVLTVLHQDWLNGKEYKCKVSNKALPAPIEKTISKAKGQPREPQVYTLPPSRDELTKNQVSLTCLVKGFYPSDIAVEWESNGQPENNYKTTPPVLDSDGSFFLYSKLTVDKSRWQQGNVFSCSVMHEALHNHYTQKSLSLSPGK

SEQ ID NO: 135 - protein, 214 aa, Artificial Sequence
  Exemplary humanized anti-SJ25C1 light chain
DILLTQSPVILSVSPGERVSFSCRASQSISNYLNWYQQRTNGSPRLLIYYTSRLHSGIPSRFSGSGSGTDFTLSINSVESEDIADYYCQQGKTVPFTFGAGTKLELKRTVAAPSVFIFPPSDEQLKSGTASVVCLLNNFYPREAKVQWKVDNALQSGNSQESVTEQDSKDSTYSLSSTLTLSKADYEKHKVYACEVTHQGLSSPVTKSFNRGEC

SEQ ID NO: 136 - protein, 459 aa, Artificial Sequence
  Exemplary humanized anti-SJ25C1 heavy chain
QVQLKQSGPGLVQPSQSLSITCTVSGFSLTSYWMHWVRQSPGKGLEWLGNIYPGSGGTNYDEKFKRRLSINKDNSKSQVFFKMNSLQSNDTAIYYCAREVTTVAYYYSMDYWGQGTLVTVSATLVTVSAASTKGPSVFPLAPSSKSTSGGTAALGCLVKDYFPEPVTVSWNSGALTSGVHTFPAVLQSSGLYSLSSVVTVPSSSLGTQTYICNVNHKPSNTKVDKKVEPKSCDKTHTCPPCPAPELLGGPSVFLFPPKPKDTLMISRTPEVTCVVVDVSHEDPEVKFNWYVDGVEVHNAKTKPREEQYNSTYRVVSVLTVLHQDWLNGKEYKCKVSNKALPAPIEKTISKAKGQPREPQVYTLPPSRDELTKNQVSLTCLVKGFYPSDIAVEWESNGQPENNYKTTPPVLDSDGSFFLYSKLTVDKSRWQQGNVFSCSVMHEALHNHYTQKSLSLSPGK

SEQ ID NO: 137 - protein, 214 aa, Artificial Sequence; identical to SEQ ID NO: 133
  Exemplary humanized anti-SJ25C1 light chain

SEQ ID NO: 138 - protein, 459 aa, Artificial Sequence
  Exemplary humanized anti-FMC63 heavy chain
QVQLKQSGPGLVQPSQSLSITCTVSGYTFTDYGVHWVRQSPGKGLEWLGVINPNNGGTDYNTPFTSRLSINKDNSKSQVFFKMNSLQSNDTAIYYCAREGNNYGSRDAMDYWGQGTLVTVSATLVTVSAASTKGPSVFPLAPSSKSTSGGTAALGCLVKDYFPEPVTVSWNSGALTSGVHTFPAVLQSSGLYSLSSVVTVPSSSLGTQTYICNVNHKPSNTKVDKKVEPKSCDKTHTCPPCPAPELLGGPSVFLFPPKPKDTLMISRTPEVTCVVVDVSHEDPEVKFNWYVDGVEVHNAKTKPREEQYNSTYRVVSVLTVLHQDWLNGKEYKCKVSNKALPAPIEKTISKAKGQPREPQVYTLPPSRDELTKNQVSLTCLVKGFYPSDIAVEWESNGQPENNYKTTPPVLDSDGSFFLYSKLTVDKSRWQQGNVFSCSVMHEALHNHYTQKSLSLSPGK

SEQ ID NO: 139 - protein, 213 aa, Artificial Sequence
  Exemplary humanized anti-FMC63 light chain
DILLTQSPVILSVSPGERVSFSCSASSGVIYMYWYQQRTNGSPRLLIKLTSNLASGIPSRFSGSGSGTDFTLSINSVESEDIADYYCQQWSSNPLTFGAGTKLELKRTVAAPSVFIFPPSDEQLKSGTASVVCLLNNFYPREAKVQWKVDNALQSGNSQESVTEQDSKDSTYSLSSTLTLSKADYEKHKVYACEVTHQGLSSPVTKSFNRGEC

SEQ ID NO: 140 - protein, 459 aa, Artificial Sequence
  Exemplary humanized anti-FMC63 heavy chain
QVQLKQSGPGLVQPSQSLSITCTVSGFSLTDYYMKWVRQSPGKGLEWLGDINPNNGGTDYNQNFKGRLSINKDNSKSQVFFKMNSLQSNDTAIYYCAREGNNYGSRDAMDYWGQGTLVTVSATLVTVSAASTKGPSVFPLAPSSKSTSGGTAALGCLVKDYFPEPVTVSWNSGALTSGVHTFPAVLQSSGLYSLSSVVTVPSSSLGTQTYICNVNHKPSNTKVDKKVEPKSCDKTHTCPPCPAPELLGGPSVFLFPPKPKDTLMISRTPEVTCVVVDVSHEDPEVKFNWYVDGVEVHNAKTKPREEQYNSTYRVVSVLTVLHQDWLNGKEYKCKVSNKALPAPIEKTISKAKGQPREPQVYTLPPSRDELTKNQVSLTCLVKGFYPSDIAVEWESNGQPENNYKTTPPVLDSDGSFFLYSKLTVDKSRWQQGNVFSCSVMHEALHNHYTQKSLSLSPGK

SEQ ID NO: 141 - protein, 213 aa, Artificial Sequence; identical to SEQ ID NO: 139
  Exemplary humanized anti-FMC63 light chain

SEQ ID NO: 142 - protein, 459 aa, Artificial Sequence
  Exemplary humanized anti-FMC63 heavy chain
QVQLKQSGPGLVQPSQSLSITCTVSGFSLTDYYMKWVRQSPGKGLEWIGDINPNNGGTDYNTPFTSRLSINKDNSKSQVFFKMNSLQSNDTAIYYCAREGNNYGSRDAMDYWGQGTLVTVSATLVTVSAASTKGPSVFPLAPSSKSTSGGTAALGCLVKDYFPEPVTVSWNSGALTSGVHTFPAVLQSSGLYSLSSVVTVPSSSLGTQTYICNVNHKPSNTKVDKKVEPKSCDKTHTCPPCPAPELLGGPSVFLFPPKPKDTLMISRTPEVTCVVVDVSHEDPEVKFNWYVDGVEVHNAKTKPREEQYNSTYRVVSVLTVLHQDWLNGKEYKCKVSNKALPAPIEKTISKAKGQPREPQVYTLPPSRDELTKNQVSLTCLVKGFYPSDIAVEWESNGQPENNYKTTPPVLDSDGSFFLYSKLTVDKSRWQQGNVFSCSVMHEALHNHYTQKSLSLSPGK

SEQ ID NO: 143 - protein, 213 aa, Artificial Sequence
  Exemplary humanized anti-FMC63 light chain
DILLTQSPVILSVSPGERVSFSCRASQSIIYMYWYQQRTNGSPRPWIYLTSNLASGIPSRFSGSGSGTDFTLSINSVESEDIADYYCQQWSSNPLTFGAGTKLELKRTVAAPSVFIFPPSDEQLKSGTASVVCLLNNFYPREAKVQWKVDNALQSGNSQESVTEQDSKDSTYSLSSTLTLSKADYEKHKVYACEVTHQGLSSPVTKSFNRGEC

SEQ ID NO: 144 - protein, 452 aa, Artificial Sequence
  Exemplary humanized anti-FMC63 heavy chain
QVQLKQSGPGLVQPSQSLSITCTVSGYSFTRYGVHWVRQSPGKGLEWLGVIHPSDSETDYNTPFTSRLSINKDNSKSQVFFKMNSLQSNDTAIYYCARIYYEEAWGQGTLVTVSATLVTVSAASTKGPSVFPLAPSSKSTSGGTAALGCLVKDYFPEPVTVSWNSGALTSGVHTFPAVLQSSGLYSLSSVVTVPSSSLGTQTYICNVNHKPSNTKVDKKVEPKSCDKTHTCPPCPAPELLGGPSVFLFPPKPKDTLMISRTPEVTCVVVDVSHEDPEVKFNWYVDGVEVHNAKTKPREEQYNSTYRVVSVLTVLHQDWLNGKEYKCKVSNKALPAPIEKTISKAKGQPREPQVYTLPPSRDELTKNQVSLTCLVKGFYPSDIAVEWESNGQPENNYKTTPPVLDSDGSFFLYSKLTVDKSRWQQGNVFSCSVMHEALHNHYTQKSLSLSPGK

SEQ ID NO: 145 - protein, 214 aa, Artificial Sequence
  Exemplary humanized anti-FMC63 light chain
DILLTQSPVILSVSPGERVSFSCRASGNIHNYLAWYQQRTNGSPRLLIKNAKTLADGIPSRFSGSGSGTDFTLSINSVESEDIADYYCQHFWSTPYTFGAGTKLELKRTVAAPSVFIFPPSDEQLKSGTASVVCLLNNFYPREAKVQWKVDNALQSGNSQESVTEQDSKDSTYSLSSTLTLSKADYEKHKVYACEVTHQGLSSPVTKSFNRGEC

SEQ ID NO: 146 - protein, 452 aa, Artificial Sequence
  Exemplary humanized anti-FMC63 heavy chain
QVQLKQSGPGLVQPSQSLSITCTVSGFSLTRYWMNWVRQSPGKGLEWLGMIHPSDSETRLNQKFKDRLSINKDNSKSQVFFKMNSLQSNDTAIYYCARIYYEEAWGQGTLVTVSATLVTVSAASTKGPSVFPLAPSSKSTSGGTAALGCLVKDYFPEPVTVSWNSGALTSGVHTFPAVLQSSGLYSLSSVVTVPSSSLGTQTYICNVNHKPSNTKVDKKVEPKSCDKTHTCPPCPAPELLGGPSVFLFPPKPKDTLMISRTPEVTCVVVDVSHEDPEVKFNWYVDGVEVHNAKTKPREEQYNSTYRVVSVLTVLHQDWLNGKEYKCKVSNKALPAPIEKTISKAKGQPREPQVYTLPPSRDELTKNQVSLTCLVKGFYPSDIAVEWESNGQPENNYKTTPPVLDSDGSFFLYSKLTVDKSRWQQGNVFSCSVMHEALHNHYTQKSLSLSPGK

SEQ ID NO: 147 - protein, 214 aa, Artificial Sequence; identical to SEQ ID NO: 145
  Exemplary humanized anti-FMC63 light chain

SEQ ID NO: 148 - protein, 452 aa, Artificial Sequence
  Exemplary humanized anti-FMC63 heavy chain
QVQLKQSGPGLVQPSQSLSITCTVSGFSLTRYWMNWVRQSPGKGLEWIGMIHPSDSETRYNTPFTSRLSINKDNSKSQVFFKMNSLQSNDTAIYYCASIYYEEYWGQGTLVTVSATLVTVSAASTKGPSVFPLAPSSKSTSGGTAALGCLVKDYFPEPVTVSWNSGALTSGVHTFPAVLQSSGLYSLSSVVTVPSSSLGTQTYICNVNHKPSNTKVDKKVEPKSCDKTHTCPPCPAPELLGGPSVFLFPPKPKDTLMISRTPEVTCVVVDVSHEDPEVKFNWYVDGVEVHNAKTKPREEQYNSTYRVVSVLTVLHQDWLNGKEYKCKVSNKALPAPIEKTISKAKGQPREPQVYTLPPSRDELTKNQVSLTCLVKGFYPSDIAVEWESNGQPENNYKTTPPVLDSDGSFFLYSKLTVDKSRWQQGNVFSCSVMHEALHNHYTQKSLSLSPGK

SEQ ID NO: 149 - protein, 214 aa, Artificial Sequence
  Exemplary humanized anti-FMC63 light chain
DILLTQSPVILSVSPGERVSFSCRASQSIHNYLAWYQQRTNGSPRLLVYNAKTLASGIPSRFSGSGSGTDFTLSINSVESEDIADYYCQHFWSTPYTFGAGTKLELKRTVAAPSVFIFPPSDEQLKSGTASVVCLLNNFYPREAKVQWKVDNALQSGNSQESVTEQDSKDSTYSLSSTLTLSKADYEKHKVYACEVTHQGLSSPVTKSFNRGEC

SEQ ID NO: 150 - protein, 12 aa, Homo sapiens
  spacer (IgG4hinge) (aa)
ESKYGPPCPPCP

SEQ ID NO: 151 - DNA, 36 bp, Homo sapiens
  spacer (IgG4hinge) (nt)
gaatctaagtacggaccgccctgccccccttgccct

SEQ ID NO: 152 - protein, 119 aa, Homo sapiens
  Hinge-CH3 spacer
ESKYGPPCPPCPGQPREPQVYTLPPSQEEMTKNQVSLTCLVKGFYPSDIAVEWESNGQPENNYKTTPPVLDSDGSFFLYSRLTVDKSRWQEGNVFSCSVMHEALHNHYTQKSLSLSLGK

SEQ ID NO: 153 - protein, 229 aa, Homo sapiens
  Hinge-CH2-CH3
ESKYGPPCPPCPAPEFLGGPSVFLFPPKPKDTLMISRTPEVTCVVVDVSQEDPEVQFNWYVDGVEVHNAKTKPREEQFNSTYRVVSVLTVLHQDWLNGKEYKCKVSNKGLPSSIEKTISKAKGQPREPQVYTLPPSQEEMTKNQVSLTCLVKGFYPSDIAVEWESNGQPENNYKTTPPVLDSDGSFFLYSRLTVDKSRWQEGNVFSCSVMHEALHNHYTQKSLSLSLGK

SEQ ID NO: 154 - protein, 282 aa, Homo sapiens
  IgD-hinge-Fc
RWPESPKAQASSVPTAQPQAEGSLAKATTAPATTRNTGRGGEEKKKEKEKEEQEERETKTPECPSHTQPLGVYLLTPAVQDLWLRDKATFTCFVVGSDLKDAHLTWEVAGKVPTGGVEEGLLERHSNGSQSQHSRLTLPRSLWNAGTSVTCTLNHPSLPPQRLMALREPAAQAPVKLSLNLLASSDPPEAASWLLCEVSGFSPPNILLMWLEDQREVNTSGFAPARPPPQPGSTTFWAWSVLRVPAPPSPQPATYTCVVSHEDSRTLLNASRSLEVSYVTDH

SEQ ID NO: 155 - protein, 335 aa, Artificial Sequence
  tEGFR
RKVCNGIGIGEFKDSLSINATNIKHFKNCTSISGDLHILPVAFRGDSFTHTPPLDPQELDILKTVKEITGFLLIQAWPENRTDLHAFENLEIIRGRTKQHGQFSLAVVSLNITSLGLRSLKEISDGDVIISGNKNLCYANTINWKKLFGTSGQKTKIISNRGENSCKATGQVCHALCSPEGCWGPEPRDCVSCRNVSRGRECVDKCNLLEGEPREFVENSECIQCHPECLPQAMNITCTGRGPDNCIQCAHYIDGPHCVKTCPAGVMGENNTLVWKYADAGHVCHLCHPNCTYGCTGPGLEGCPTNGPKIPSIATGMVGALLLLLVVALGIGLFM

SEQ ID NO: 156 - protein, 357 aa, Artificial Sequence
  tEGFR
MLLLVTSLLLCELPHPAFLLIPRKVCNGIGIGEFKDSLSINATNIKHFKNCTSISGDLHILPVAFRGDSFTHTPPLDPQELDILKTVKEITGFLLIQAWPENRTDLHAFENLEIIRGRTKQHGQFSLAVVSLNITSLGLRSLKEISDGDVIISGNKNLCYANTINWKKLFGTSGQKTKIISNRGENSCKATGQVCHALCSPEGCWGPEPRDCVSCRNVSRGRECVDKCNLLEGEPREFVENSECIQCHPECLPQAMNITCTGRGPDNCIQCAHYIDGPHCVKTCPAGVMGENNTLVWKYADAGHVCHLCHPNCTYGCTGPGLEGCPTNGPKIPSIATGMVGALLLLLVVALGIGLFM

SEQ ID NO: 157 - protein, 27 aa, Homo sapiens
  CD28 (amino acids 153-179 of Accession No. P10747)
FWVLVVVGGVLACYSLLVTVAFIIFWV

SEQ ID NO: 158 - protein, 66 aa, Homo sapiens
  CD28 (amino acids 114-179 of Accession No. P10747)
IEVMYPPPYLDNEKSNGTIIHVKGKHLCPSPLFPGPSKPFWVLVVVGGVLACYSLLVTVAFIIFWV

SEQ ID NO: 159 - protein, 41 aa, Homo sapiens
  CD28 (amino acids 180-220 of P10747)
RSKRSRLLHSDYMNMTPRRPGPTRKHYQPYAPPRDFAAYRS

SEQ ID NO: 160 - protein, 41 aa, Homo sapiens
  CD28 (LL to GG)
RSKRSRGGHSDYMNMTPRRPGPTRKHYQPYAPPRDFAAYRS

SEQ ID NO: 161 - protein, 42 aa, Homo sapiens
  4-1BB (amino acids 214-255 of Q07011.1)
KRGRKKLLYIFKQPFMRPVQTTQEEDGCSCRFPEEEEGGCEL

SEQ ID NO: 162 - protein, 112 aa, Homo sapiens
  CD3 zeta
RVKFSRSADAPAYQQGQNQLYNELNLGRREEYDVLDKRRGRDPEMGGKPRRKNPQEGLYNELQKDKMAEAYSEIGMKGERRRGKGHDGLYQGLSTATKDTYDALHMQALPPR

SEQ ID NO: 163 - protein, 112 aa, Homo sapiens
  CD3 zeta
RVKFSRSAEPPAYQQGQNQLYNELNLGRREEYDVLDKRRGRDPEMGGKPRRKNPQEGLYNELQKDKMAEAYSEIGMKGERRRGKGHDGLYQGLSTATKDTYDALHMQALPPR

SEQ ID NO: 164 - protein, 112 aa, Homo sapiens
  CD3 zeta
RVKFSRSADAPAYKQGQNQLYNELNLGRREEYDVLDKRRGRDPEMGGKPRRKNPQEGLYNELQKDKMAEAYSEIGMKGERRRGKGHDGLYQGLSTATKDTYDALHMQALPPR